European Patent Specification EP 3 470 420 B1, published October 22, 2025. Title: Methods of Modulating Seed and Organ Size in Plants. Applicant: Institute of Genetics and Developmental Biology Plant Bioscience Limited. Application EP. The sequence listing filed with the application follows.

SEQUENCE LISTING (91 sequences)

SEQ ID NO: 1 - protein, 43 aa, Artificial sequence
  Synthetic sequence: RING domain
  VARIANT (2)..(3): Xaa is any amino acid
  VARIANT (5)..(15): Xaa is any amino acid
  VARIANT (18)..(21): Xaa is any amino acid
  VARIANT (23)..(24): Xaa is any amino acid
  VARIANT (26)..(32): Xaa is any amino acid
  VARIANT (33)..(33): Xaa is His, Asn or Thr
  VARIANT (34)..(39): Xaa is any amino acid
  VARIANT (41)..(42): Xaa is any amino acid
CXXCXXXXXXXXXXXCCXXXXCXXCXXXXXXXXXXXXXXCXXC

SEQ ID NO: 2 - protein, 43 aa, Artificial sequence
  Synthetic sequence RING domain
  VARIANT (7)..(7): Xaa is Tyr or Phe
  VARIANT (15)..(15): Xaa is Lys or Arg
  VARIANT (18)..(18): Xaa is Ser, Met, Thr or Ala
  VARIANT (20)..(20): Xaa is Gly or Ser
  VARIANT (28)..(28): Xaa is Gln or Arg
  VARIANT (31)..(31): Xaa is Pro, Asn, Ser, Val, Thr or Asn
  VARIANT (32)..(32): Xaa is Thr or Pro
  VARIANT (33)..(33): Xaa is His, Asn or Thr
  VARIANT (34)..(34): Xaa is Thr or Ser
  VARIANT (35)..(35): Xaa is Ala, Thr or Cys
  VARIANT (36)..(36): Xaa is Arg, Gln or Lys
  VARIANT (42)..(42): Xaa is Phe or Tyr
CPICFLXYPSLNRSXCCXKXICTECFLXMKXXXXXXPTQCPXC

SEQ ID NO: 3 - protein, 43 aa, Brachypodium distachyon
CPICFLYYPSLNRSKCCSKGICTECFLQMKPTHTARPTQCPFC

SEQ ID NO: 4 - protein, 43 aa, Hordeum vulgare; identical to SEQ ID NO: 3

SEQ ID NO: 5 - protein, 43 aa, Zea mays; identical to SEQ ID NO: 3

SEQ ID NO: 6 - protein, 43 aa, Sorghum bicolor; identical to SEQ ID NO: 3

SEQ ID NO: 7 - protein, 43 aa, Oryza sativa
CPICFLYYPSLNRSKCCSKGICTECFLQMKPTHTAQPTQCPFC

SEQ ID NO: 8 - protein, 43 aa, Populus trichocarpa
CPICFLYYPSLNRSRCCMKGICTECFLQMKNPNSTRPTQCPFC

SEQ ID NO: 9 - protein, 43 aa, Carica papaya; identical to SEQ ID NO: 8

SEQ ID NO: 10 - protein, 43 aa, Ricinus communis; identical to SEQ ID NO: 8

SEQ ID NO: 11 - protein, 43 aa, Arabidopsis thaliana
CPICFLYYPSLNRSRCCMKSICTECFLQMKNPNSARPTQCPFC

SEQ ID NO: 12 - protein, 43 aa, Brassica napus; identical to SEQ ID NO: 11

SEQ ID NO: 13 - protein, 43 aa, Arabidopsis thaliana
CPICFLYYPSLNRSRCCMKSICTECFLRMKSPNSAQPTQCPFC

SEQ ID NO: 14 - protein, 43 aa, Glycine max
CPICFLYYPSLNRSRCCTKSICTECFLQMKVPNSTRPTQCPFC

SEQ ID NO: 15 - protein, 43 aa, Sorghum bicolor
CPICFLFYPSLNRSKCCAKGICTECFLQMKSPTSCRPTQCPYC

SEQ ID NO: 16 - protein, 43 aa, Brachypodium distachyon; identical to SEQ ID NO: 15

SEQ ID NO: 17 - protein, 43 aa, Zea mays
CPICFLFYPSLNRSKCCAKGICTECFLQMKSPTSCKPTQCPYC

SEQ ID NO: 18 - protein, 43 aa, Oryza sativa
CPICFLFYPSLNRSKCCAKGICTECFLQMRTPTSCRPTQCPYC

SEQ ID NO: 19 - protein, 43 aa, Vitis vinifera
CPICFLFYPSLNRSRCCTKGICTECFLQMKNPNSTRPTQCPYC

SEQ ID NO: 20 - protein, 423 aa, Populus trichocarpa
MGNKLGRRRQVVDERYTRPQGLYVHKDVDHKKLRKLILESKLAPCFPGDEDSCNDHEECPICFLYYPSLNRSRCCMKGICTECFLQMKNPNSTRPTQCPFCKTSNYAVEYRGVKTKEEKGLEQIEEQRVIEAKIRMRQQELQDEEERMQKRLDVSSSSANIEPGELECGPTTVPSDTTPVESGEIVSSQYSSRRPPHAGANRDDEFDLDLEDIMVMEAIWLSIQENGRQKNPLCGDAAPPAQYTMEARYVTPAMAPPLAGSSSSPSGGLACAIAALAERQQTGGESIVHNSGNMPSFNMLPSTSSFYNRLEQDADNYSPAQSSSNVLPDCRMIVTRDDGEWGADRGSDAAEAGTSYASSETAEDAGGISSLLPPPPPTDEIGGSFQNVSGPIPESFEEQMMLAMAVSLAEARAMTSGPQSAWQ

SEQ ID NO: 21 - protein, 420 aa, Ricinus communis
MGNKLGRRRQVVDERYTRPQGLYVHKDVDHKKLRKLILESKLAPCYPGDDEFGNDHEECPICFLYYPSLNRSRCCMKGICTECFLQMKNPNSTRPTQCPFCKTTNYAVEYRGVKTKEEKGMEQIEEQRVIEAKIRMRQQELQDEEERMQKRLELSSSSSSIAPGEVECGSAAVQSFRSPLEAEGSIPSQFSIRHPPHYRANRDDEFDLDLEDIMVMEAIWLSIQENGRQKNPIYTDAASSENYAVQGHYALQAMPPVTESSSSPSGGLACAIAALAERQQTGGESFAHNNENVAACNMLPGGSSFYNRMDQDAENYSPAQGSNNMLSDCRMARDDVQWVADRGSDAAEAGTSYASSETTEDSDGISVVLPPPPLPPPDEIVGSDSGMIVPESFEEQMMLAMAVSLAEAQAMTGGAGSAWQ

SEQ ID NO: 22 - protein, 423 aa, Vitis vinifera
MGNKLGRRRQVVEDKYTRPQGLYQHKDVDHKKLRKLILDSKLAPCYPGDEEATNDFEECPICFLFYPSLNRSRCCTKGICTECFLQMKNPNSTRPTQCPYCKTANYAVEYRGVKTKEEKGMEQIEEQRVIEAKIRMRQKEIQDEEERMQKRQEISSSSSILAQGEVEYSTTAVPSFRSPVEGDEIDSSQDPRAASMIIQTLPPRQNRDEEFDLDLEDIMVMEAIWLSIQDNGRHRNPLYGDTTTAEQYVTEEHYVLPAMAPQVESSSSPSGGLACAIAALAERQQMGGESSTNYNGNMPAFNMPPGSSRFSNRVEQYPENYPPIESSMDALPDGGLAVTKDDGEWGVDRGSEVAEAGTSYASSDATDEAGGVAALPPTDEAEGSFQNVGGPIVPESFEEQMMLAMAVSLAEARARTSTQGVWQ

SEQ ID NO: 23 - protein, 431 aa, Glycine max
MGNKLGRRRQVVDEKYTRPQGLYNHKDVDHKKLRKLILESKLAPCYPGDEETAYDREECPICFLYYPSLNRSRCCTKSICTECFLQMKVPNSTRPTQCPFCKTANYAVEYRGVKSKEEKGLEQIEEQRVIEAKIRMRQQELQDEEERMHKRLEMSSSNVNVAVADVEYSSNAVSSSSVSVVENDEIVSSQDSCATSVVRANATTRTNRDDEFDVDLEDIMVMEAIWLSIQENGRRRNLSFVDATSGHYVADGRYVSSVSSVSSVMGPPTGSSSSPSGGLACAIAALAERQQMAGESSMSLTNENMPSFNTLPGSRRFYNRLGRDMANYPPGDNLNEEPLDEAVTMTRSHGEWDMDHGTQLTETATSYTNSVAAEDRGELSSLPRSDDNDGSLQSATEPIVPESFEEQMMLAMAVSLAEARAMSSGQSASWQ

SEQ ID NO: 24 - protein, 401 aa, Arabidopsis thaliana
MGNKLGRKRQVVEERYTKPQGLYVNKDVDVKKLRKLIVESKLAPCYPGDDESCHDLEECPICFLYYPSLNRSRCCMKSICTECFLQMKNPNSARPTQCPFCKTPNYAVEYRGVKSKEEKGIEQVEEQRVIEAKIRMRQKEMQDDEEKMQKRLESCSSSTSAMTGEMEYGSTSAISYNSLMDDGEIAPSQNASVVRQHSRPRGNREDEVDVDLEELMVMEAIWLSVQETGTQRNSASGEITSSRQYVTDNHSYVSSPPRVTPIVEPATPSSSSGGLSCAISALAERQMVGESSSHNHNHNVNVSSYSMLPGNCDSYYDIEQEVDGIDNHHHHRHHYEMGETGSSNSYVSSYMTGEGFHNFPPPPPLVIVPESFEEQMMMAMAVSMAEVHATTTCAPTEVTWQ

SEQ ID NO: 25 - protein, 424 aa, Triticum aestivum
MGNRIGGRRKAGVEERYTRPQGLYEHRDIDQKKLRKLILEAKLAPCYPGADDAAGGDLEECPICFLYYPSLNRSKCCSKGICTECFLQMKPTHTARPTQCPFCKTPNYAVEYRGVKTKEERSIEQFEEQKVIEAQMRMRQQALQDEEDKMKRKQSRCSSSRTIAPTTEVEYRDICSTSYSVPSYQCTEQETECCSSEPSCSAQANMRSFHSRHTRDDNIDMNIEDMMVMEAIWRSIQEQGSIGNPACGSFMPFEQPTCERQAFVAAPPLEIPHPGGFSCAVAAMAEHQPSSMDFSYMTGSSAFPVFDMFRRPCNIAGGSMCAVESSPDSWSGIASSCSRREVVREEGECSTDHWSEGAEAGTSYAGSDIVVDAGTTPPLPVTDNYSMVASHFRPESIEEQMMYSMAVSLAEAHGRTHTQGLAWL

SEQ ID NO: 26 - protein, 424 aa, Hordeum vulgare
MGNRIGGRRKAGVEERYTRPQGLYEHRDIDQKKLRKLILETKLAPCYPGADDAAGADLEECPICFLYYPSLNRSKCCSKGICTECFLQMKPTHTARPTQCPFCKTPNYAVEYRGVKTKEERSIEQFEEQKVIEAQMRMRQQALQDEEDKMRRKQSRCSSSRTIAPTTEVEYRDICSTSYSAPPYRCTEQETECCSSEPSCSAQANMRSFHSRHTRDGNIDMNIEDMMVMEAIWRSIQEQGSIGNPACGSFMPFEQPTRERQAFVAASPLEIPHPGGFSCAVAAMTEHQPSSMDFSYMTGSSAFPVFDMFRRPCNIAGGSLRAVESSLDSWSGIAPSGTRREMVREEGECSIDHWSEGAEAGTSYAGSDIMADAGTMPPLPFADNYSMAASHFRPESIEEQMMYSMAVSLAEAHGRTHTQGLTWL

SEQ ID NO: 27 - protein, 423 aa, Brachypodium distachyon
MGNRIGGRRKAGVEERYTRPQGLYEHRDIDQKKLRKLILEAKLAPCYPGADDAAGGDLEECPICFLYYPSLNRSKCCSKGICTECFLQMKPTHTARPTQCPFCKTPNYAVEYRGVKTKEERSIEQLEEQKVIEAQMRMRQQALQDEEDKMKRKQSRCSSSRTIAPTTEVEYRDICSTSYSVPSYQCTEQEAECCSSEPSCSAQSNMRPVHSRHNRDDNIGMNIEEMMVMEAIWRSIQEQGSMGNPVCGNFMPVIEPPSRERQAFVPAPLEIPHPGGFSCAVASMAEHQPPSMDFSYMAGNSAFPVFDMFRRQCNISGGSMCAVDSSPDSWSGIPPSCSREMIREEGECSTDHWSEGAEAGTSYAGSDIVADAGTMQQLPFAENYNMAPSHFRPESIEEQMMYSMTVSLAEAHGRTHSQGLAWL

SEQ ID NO: 28 - protein, 423 aa, Oryza sativa
MGNRIGGRRKAGVEERYTRPQGLYEHRDIDQKKLRKLILEAKLAPCYMGADDAAAAADLEECPICFLYYPSLNRSKCCSKGICTECFLQMKPTHTAQPTQCPFCKTPSYAVEYRGVKTKEERSIEQFEEQKVIEAQMRMRQQALQDEEDKMKRKQNRCSSSRTITPTKEVEYRDICSTSFSVPSYRCAEQETECCSSEPSCSAQTSMRPFHSRHNRDDNIDMNIEDMMVMEAIWRSIQGSIGNPVCGNFMPVTEPSPRERQPFVPAASLEIPHGGGFSCAVAAMAEHQPPSMDFSYMAGSSAFPVFDMFRRPCNIAGGSMCNLESSPESWSGIAPSCSREVVREEGECSADHWSEGAEAGTSYAGSDIVADAGTMPQLPFAENFAMAPSHFRPESIEEQMMFSMALSLADGHGRTHSQGLAWL

SEQ ID NO: 29 - protein, 428 aa, Sorghum bicolor
MGNRKGGRPKSGGEKRFTPPQGLYEHKDIDQKKLRKLILEAKLAPCYPGADDAAAAGGDLEECPICFLYYPSLNRSKCCSKGICTECFLQMKPTHTARPTQCPFCKTPNYAVEYRGVKTKEERSIEQFEEQKVIEAQLRMRQKELQDEEAKMKRKQSRCSSSRTVTPTTEVEYRDICSTSFSVPSYQCTEQGNECCSSEPSCSSQANMRPFHSRHNRDDNVDVNLEDMMVMEAIWRSIQEQGHLVNPVCGSYFPVIEPPSRERQAFLPAAPLEMPHPGGYSCAVAALAEHQPASMDFSYMAGSSTYPVFDMIRRPCNMSSGSLCGVENSSLDTWSGIAPSCSREVVREEGECSTDHWSEGAEAGTSYAGSDIMADTGTMQPLPFAENFTMAPSHFRPESIEEQMMFSMAVSLAEAHHGRTQAQGLAWL

SEQ ID NO: 30 - protein, 431 aa, Zea mays
MGNRIGGRRKPGVEERFTRPQGLYEHKDIDQKKLRKLILEAKLAPCYPGADDAAAGGGDLDLEECPICFLYYPSLNRSKCCSKGICTECFLQMKPTHTARPTQCPFCKTANYAVEYRGVKTKEERSIEQFEEQKVIEAQLRMRQKELQDEEAKMKRKQSRCSSSRTVTPTTEVEYRDICSTSFSVPSYQRTEQGNECCSSEPSCSSQANMRPFHSRHNRDDNVDMNLEDMMVMETIWRSIQQEQGHLVNPVCGSYFPVIEPPSRERQAFVPAAPLEMPHPGGYSCAVAALAEHQAPSMDFSYMSGSSTYPVFDMIRRPCNMSSGSPCGAENSSLDTWSGIAPSCSREVVRDEGECSADHWSEGAEAGTSYAGSDIMADAGAMQPLPFAENFAMGPSHFRPESVEEQMMFSMAVSLAEAHHGRTQAQGLAWL

SEQ ID NO: 31 - protein, 424 aa, Triticum aestivum
MGNRIGGRRKAGVEERYTRPQGLYEHRDIDQKKLRKLILEAKLAPCYPGADDAAGGDLEECPICFLYYPSLNRSKCCSKGICTECFLQMKPTHTARPTQCPFCKTPNYAVEYRGVKTKEERSIEQFEEQKVIEAQMRVRQQALQDEEDKMKRKQSRCSSSCKTPNYAVEYRGVKTKEERSIEQFEEQKVIEAQMRVRQQALQDEEDKMKRKQSRCSSSMDMNIEDMMVMEAIWRSIQEQGSIGNPSCGSFMPFEQPTRERQAFVAAPPLEMPHPGGMDMNIEDMMVMEAIWRSIQEQGSIGNPSCGSFMPFEQPTRERQAFVAAPPLEMPHPGGPSCSRREVVREEGECSTDHLSEGAEAGTSYAGSDIVVDAGTMLPLPFADNYSMVASHFRPESIEEQMMYSMAVSLAEAHGRTHSQGLAWL

SEQ ID NO: 32 - protein, 398 aa, Brachypodium distachyon
MGNQGLYPHPDIDLKKLRRLIVEAKLAPCHPGSDDPRADLDECPICFLFYPSLNRSKCCAKGICTECFLQMKSPTSCRPTQCPYCKMLNYAVEYRGVKTKEEKGVEQLEEQRVIEAQIRMRHQEIKDDAERLKNKQTATLSDVITTPQVECCEAGGTSTPAASSAQGNDALLSQVQHSELLLKNSERLKQMRENNFDVDLEEVMLMEAIWLSVQDASGNPGITGAAPPTIPPRSYDTSVTASAEAAPSGGFACAVAALAEQQHMLVGSSIPATCQASKHDTLSRSDRSFTEDLSIAGSSSSGTRVDESSINRTRQTREGAEHSNNDRWSEVADASTSCAGSDITREAGAANLVASDGSSIGSGNIPDSFEDQMMLAISLSLVDARAMASSPGPGLTWQ

SEQ ID NO: 33 - protein, 414 aa, Oryza sativa
MGNQVGGRRRRRPAVEERYTRPQGLYPHPDIDLKKLRRLIVEAKLAPCFPGSDDPRADLEECPICFLFYPSLNRSKCCAKGICTECFLQMRTPTSCRPTQCPYCKMASYAVEYRGVKTKEEKGTEQIEEQRVIEAQIRMRQQELQDDAERMKKKQAAALTDVVTTAQVEHCDTGGASTTVKSSGQGSDMLSSQVQHAELLLKTSERLKQMRNNNFDMDPDEVMLVEALWLSLQDQEASGNPTCGNTVSSVHPPRSFEGSMTIPAEAASSSSAFACAVAALAEQQQMYGEASSTATCHTSRCDILSRSDRSFTEDLSINGSGSSGARSEEPSSNKMHQTREGMEYSNERWSEMAEASSSFTGSDLTTEAGAANSGGSDTGAGSIPDSFEEQMMLAMALSLADARAKASSPGLTWR

SEQ ID NO: 34 - protein, 419 aa, Zea mays
MGNQVGGRRRRRPPVDERYTRPQGLYPHPDIDLRKLRRLILEAKLAPCHPGADDARADLDECPICFLFYPSLNRSKCCAKGICTECFLQMKSPTSCKPTQCPYCKTLNYAVEYRGVKTKEEKGIEQLEEQRVIEAQIRMRQQEVQDDAERMKNKRTATLGDVVASAQVDSCNTDGASTAVANSPRGNDVLSSEVQHSELISRNSEAFKQMRGNNFEVDLEEVMLMEAIWLSIQDQEALGNPGCVSTTPSSIPSRPFDDGDMTTTAEAASSGGFACAVAALAEQQHMHGESSSASPCQTIRFGTLSRPDRSTTQDLSVAGSSSSDSRVEEPPTSNTHRTIEAAEYSNSNVQWSEVAEAGTSIAESDGTVEAGVDNSSTSAGSNIDSVSVPDSFEEQMMLAMALSLVDARARAGSPGLAWR

SEQ ID NO: 35 - protein, 418 aa, Sorghum bicolor
MGNQVGGRRRRRPAVDERYTQPQGLYPHPDIDLRKLRRLILEAKLAPCHPGADDARADLDECPICFLFYPSLNRSKCCAKGICTECFLQMKSPTSCRPTQCPYCKTLNYAVEYRGVKTKEEKGIEQLEEQRVIEAQIRMRQKELQDDAERMKNKQTATLGDIVASAQVDSCNTDGASTGAASSPQGSDAISSEVQHSELILRNSEAFKQMRGNNFDVDLEEVMLMEAIWLSIQDQEALGNSGCVSTTPSSIPSRPFDGAMTTTPEAASSGGFAFAVAALAEQQHMHGESSSASACQTPRFDILSRSDRSSTEDLSVVGSSSSDSRVEEPSSSSTHRTIEGSEYSNSNGRWSEVAEAGTSIAEADVIVEAGVGNSSTSVGSNIGSSSVPDSFEEQMMLAMALSLVDARSRAGSPGLAWR

SEQ ID NO: 36 - protein, 27 aa, Artificial sequence
  Synthetic sequence: DA2 polypeptide first consensus domain
  VARIANT (2)..(2): May be present or absent; if present, Xaa is Gln
  VARIANT (6)..(6): Xaa is Pro, Met, Asn, Val, Gln, Leu, Val or Glu
  VARIANT (7)..(7): Xaa is His, Ser or Asn
  VARIANT (8)..(8): Xaa is Pro, Lys or Arg
  VARIANT (10)..(10): Xaa is Ile or Val
  VARIANT (12)..(12): Xaa is Leu, Ile, His, Val or Gln
  VARIANT (13)..(13): Xaa is Lys or Arg
  VARIANT (16)..(16): Xaa is Arg or Lys
  VARIANT (17)..(17): Xaa is Arg or Lys
  VARIANT (20)..(20): Xaa is Val or Leu
  VARIANT (21)..(21): Xaa is Glu or Asp
  VARIANT (22)..(22): Xaa is Ala, Ser or Thr
QXGLYXXXDXDXXKLXXLIXXXKLAPC

SEQ ID NO: 37 - protein, 36 aa, Artificial sequence
  Synthetic sequence: DA2 polypeptide second consensus domain
  VARIANT (1)..(1): Xaa is Asn or Ser
  VARIANT (9)..(9): Xaa is Val or Gly
  VARIANT (11)..(11): Xaa is Thr or Ser
  VARIANT (15)..(15): Xaa is Lys or Arg
  VARIANT (16)..(16): Xaa is Gly or Ser
  VARIANT (17)..(17): Xaa is Val, Thr, Ile, Phe, Leu or Met
  VARIANT (20)..(20): Xaa is Leu, Ile, Val or Phe
  VARIANT (24)..(24): Xaa is Arg, Leu or Lys
  VARIANT (29)..(29): Xaa is Gln or Lys
  VARIANT (30)..(30): Xaa is Ile or Met
  VARIANT (34)..(34): Xaa is His or Gln
  VARIANT (35)..(35): Xaa is Lys or Gln
  VARIANT (36)..(36): Xaa is Glu or Ala
XYAVEYRGXKXKEEXXXEQXEEQXVIEAXXRMRXXX

SEQ ID NO: 38 - protein, 66 aa, Artificial sequence
  Synthetic sequence: LIM domain
  VARIANT (2)..(3): Xaa is any amino acid
  VARIANT (5)..(27): Xaa at positions 5 to 27 is any amino acid and up to seven of them may be absent; represents a range of 16 - 23 amino acids.
  VARIANT (28)..(28): Xaa is His or Cys
  VARIANT (29)..(32): Xaa at positions 29 to 32 is any amino acid and any two of them may be absent; represents a string of 2 or 4 amino acids.
  VARIANT (33)..(33): Xaa is Cys, His or Glu
  VARIANT (34)..(35): Xaa is any amino acid
  VARIANT (37)..(38): Xaa is any amino acid
  VARIANT (40)..(60): Xaa at positions 40 to 60 is any amino acid and up to seven of them may be absent; represents a range of 14 - 21 amino acids.
  VARIANT (61)..(61): Xaa is Cys or His
  VARIANT (62)..(64): Xaa at positions 62 - 64 is any amino acid and any one or two of them may be absent; represents a string of 2 or 1 or 3 amino acids.
  VARIANT (65)..(65): Xaa is Cys, His, Asp or Glu
  VARIANT (66)..(66): Xaa is any amino acid
CXXCXXXXXXXXXXXXXXXXXXXXXXXXXXXXXXXCXXCXXXXXXXXXXXXXXXXXXXXXXXXXXX

SEQ ID NO: 39 - protein, 63 aa, Artificial sequence
  Synthetic sequence: LIM domain
  VARIANT (2)..(3): Xaa is any amino acid
  VARIANT (5)..(27): Xaa at positions 5 - 27 is any amino acid and up to seven of them may be absent; represents a range of 16 - 23 amino acids.
  VARIANT (29)..(30): Xaa is any amino acid
  VARIANT (32)..(33): Xaa is any amino acid
  VARIANT (35)..(36): Xaa is any amino acid
  VARIANT (38)..(58): Xaa at positions 38 to 58 is any amino acid and up to seven of them may be absent; represents a range of 14 - 21 amino acids.
  VARIANT (60)..(61): Xaa is any amino acid
  VARIANT (63)..(63): Xaa is any amino acid
CXXCXXXXXXXXXXXXXXXXXXXXXXXHXXCXXCXXCXXXXXXXXXXXXXXXXXXXXXHXXCX

SEQ ID NO: 40 - protein, 53 aa, Arabidopsis thaliana
CAGCNMEIGHGRFLNCLNSLWHPECFRCYGCSQPISEYEFSTSGNYPFHKACY

SEQ ID NO: 41 - protein, 504 aa, Setaria italica
MGWLSKIFKGSVNRVSRGHYNGNSHEGYSTQHTKSYGAHGNEDEDMDHAIALSLSEQDQRKGKAIDTEHHLDEDEQLARALQENTSPTLDEDEQLARALQESMNDEHPPRQHIPIEDVHSESAPASSLPPYVFPTNGSRVCAGCKTPIGQGRFLSCMDSVWHPQCFRCYGCDIPISEYEFAVHEDHAYHRSCYKERFHPKCDVCNSFIPTNKNGLIEYRAHPFWMQKYCPSHENDGTPRCCSCERMEPKHSQYITLDDGRRLCLECLHTAIMDTNECQPLYIDIQEFYEGMNMKVEQQVPLLLVERQALNEAMEAEKIGHHLPETRGLCLSEEQIVRTILRRPIIGPGNRIIDMITGPYKLVRRCEVTAILILYGLPRLLTGSILAHEMMHAYLRLKGYRTLSPEVEEGICQVLAHLWLESEITSGSGSMATTSAASSSSSTSSSSKKGAKTEFEKRLGEFFKHQIETDPSVAYGDGFRAGMRAVERYGLRSTLDHIKLTGSFP

SEQ ID NO: 42 - protein, 487 aa, Brachypodium distachyon
MGWLNKIFKGSVNRVSRGNYDGNWHDGNSSENIRGAYDESDNEDIDRAIALSLAEEDPNKGKAIIDPDYSLEEDEQLARALHESLNTGSPPHQNVPVVDVPSERVPTREPPPPVFLSSGFRACAGCNNPIGNGRFLSCMDSVWHPQCFRCFACNKPISEYEFAMHENQPYHKSCYKDFFHPKCDVCKDFIPTNKDGLIEYRAHPFWMQKYCPSHEDDGTPRCCSCERMEPTDIKYIRLDDGRKLCLECLTSATMDSPECQHLYMDIQEFFEGLNMKVEQQVPLLLVERQALNEALEAEKSGHHLPETRGLCLSEEQIVRTILRRPTIGPGNRIIDMITGPYKLVRRCEVTAILILYGLPRLQTGSILAHEMMHAYLRLKGYRSLSPQVEEGICQVLSHMWLESEIIAGASGNTASTSVPSSSSAPTSSKKGAKTEFEKRLGAFIKNQIETDSSVEYGDGFRAGNRAVERYGLRSTLDHMKITGSFPY

SEQ ID NO: 43 - protein, 514 aa, Brassica rapa
MGWLNKIFKGSNQRHPLGNEHYHHNGGYYENYPHEHSEPSAETDADHTQEPSTSEEETWNGKENEEVDRVIALSILEEENQRPETNTGAWKHAMMDDDEQLARAIQESMIARNGTTYDFGNAYGNGHMHGGGNVYDNGDIYYPRPIAFSMDFRICAGCNMEIGHGRYLNCLNALWHPQCFRCYGCSHPISEYEFSTSGNYPFHKACYRERFHPKCDVCSLFISTNHAGLIEYRAHPFWVQKYCPSHEHDATPRCCSCERMEPRNTGYFELNDGRKLCLECLDSSVMDTFQCQPLYLQIQEFYEGLNMTVEQEVPLLLVERQALNEAREGERNGHYHMPETRGLCLSEEQTVRTVRKRSKGNWSGNMITEQFKLTRRCEVTAILILFGLPRLLTGSILAHEMMHAWMRLKGFRPLSQDVEEGICQVMAHKWLEAELAAGSRNSNAASSSSSSYGGVKKGPRSQYERKLGEFFKHQIESDASPVYGDGFRAGRLAVNKYGLWRTLEHIQMTGRFPV

SEQ ID NO: 44 - protein, 532 aa, Brassica rapa
MGWFNKIFKGSTQRFRLGNDHDHNGYYQSYPHDEPSADTDPDPDPDPDETHTQEPSTSEEDTSGQENEDIDRAIALSLIENSQGQTNNTCAANAGKYAMVDEDEQLARAIQESMVVGNTPRQKHGSSYDIGNAYGAGDVYGNGHMHGGGNVYANGDIYYPRPTAFPMDFRICAGCNMEIGHGRYLNCLNALWHPECFRCYGCRHPISEYEFSTSGNYPFHKACYRERYHPKCDVCSLFIPTNHAGLIGYRAHPFWVQKYCPSHEHDATPRCCSCERMEPRNTGYVELNDGRKLCLECLDSAVMDTFQCQPLYLQIQEFYEGLFMKVEQDVPLLLVERQALNEAREGEKNGHYHMPETRGLCLSEEQTVSTVRKRSKHGTGNWAGNMITEPYKLTRQCEVTAILILFGLPRLLTGSILAHEMMHAWMRLKGFRTLSQDVEEGICQVMAHKWLEAELAAGSRNSNVASSSSSRGVKKGPRSQYERKLGEFFKHQIESDASPVYGDGFRAGRLAVNKYGLPKTLEHIQMTGRFPV

SEQ ID NO: 45 - protein, 532 aa, Arabidopsis thaliana
MGWFNKIFKGSNQRLRVGNNKHNHNVYYDNYPTASHDDEPSAADTDADNDEPHHTQEPSTSEDNTSNDQENEDIDRAIALSLLEENQEQTSISGKYSMPVDEDEQLARALQESMVVGNSPRHKSGSTYDNGNAYGAGDLYGNGHMYGGGNVYANGDIYYPRPITFQMDFRICAGCNMEIGHGRFLNCLNSLWHPECFRCYGCSQPISEYEFSTSGNYPFHKACYRERYHPKCDVCSHFIPTNHAGLIEYRAHPFWVQKYCPSHEHDATPRCCSCERMEPRNTRYVELNDGRKLCLECLDSAVMDTMQCQPLYLQIQNFYEGLNMKVEQEVPLLLVERQALNEAREGEKNGHYHMPETRGLCLSEEQTVSTVRKRSKHGTGKWAGNITEPYKLTRQCEVTAILILFGLPRLLTGSILAHEMMHAWMRLKGFRTLSQDVEEGICQVMAHKWLDAELAAGSTNSNAASSSSSSQGLKKGPRSQYERKLGEFFKHQIESDASPVYGDGFRAGRLAVHKYGLRKTLEHIQMTGRFPV

SEQ ID NO: 46 - protein, 478 aa, Theobroma cacao
MDWIKKIFKGCAHKFSEGHHHGNYVEDPHPQFNAPSVSGDAWQELENEDVDRAIALSLLGESQKGRKVIDDEYQLEEDEQLARALQESLNFEPPPQYENANMYQPMPVHFPMGYRICAGCNTEIGHGRFLNCLNAFWHPECFRCHACNLPISDYEFSMSGNYRFHKSCYKERYHPKCDVCNDFIPTNPAGLIEYRAHPFWIQKYCPSHEHDSTPRCCSCERMEPQDTGYVALNDGRKLCLECLDSAVMDTKQCQPLYLDILEFYEGLNMKVEQQVPLLLVERQALNEAREGEKNGHYHMPETRGLCLSEEQTVSTILRQPRFGTGNRAMDMITEPCKLTRRCEVTAILILYGLPRLLTGSILAHEMMHAWMRLQGFRTLSQDVEEGICQVLAHMWLLTQLEYASSSNVASASSSASSRLQKGKRPQFEGKLGEFFKHQIESDTSPVYGDGFRAGHQAVYKYGLRRTLEHIRMTGRFPY

SEQ ID NO: 47 - protein, 474 aa, Glycine max
MGWLSRIFKGSDHNKLSEGHYYKEDAGYYLPSTSGVTNNQNENEDIDRAIALSLVEESRRANNNVNGERILSLQTLLEEDEQLARAIEQSLNLESPPRYGNENMYQPPIQYFPLGICAGCYTEIGFGRYLNCLNAFWHPECFRCRACNLPISDYEFSTSGNYPYHKSCYKESYHPKCDVCKHFIPTNPAGLIEYRAHPFWIQKYCPTHEHDGTPRCCSCERMESQEAGYIALKDGRKLCLECLDSSIMDTNECQPLHADIQRFYDSLNMKLDQQIPLLLVERQALNEAREGEKNGHYHMPETRGLCLSEELSTFSRRPRLGTAMDMRAQPYRPTTRCDVTAILVLYGLPRLLTGSILAHEMMHAWLRLKGYRTLSQDVEEGICQVLAHMWLESELSSASGSNFVSASSSSASHTSRKGKRPQFERKLGEFFKHQIESDISPVYGDGFRAGQKAVRKYGLQRTLHHIRMTGTFPY

SEQ ID NO: 48 - protein, 478 aa, Glycine max
MGWLSRIFKGSDHNKLSEGHYYKEDAGYYLPSTSGVTNDAWNQSQNQNENEDIDRAIALSLVEETQKANNNVNDYRSQLEEDEQLARAIEQSLNLESPPRYGNENMYQPPIQYFPMGSRICAGCYTEIGYGRYLNCLNAFWHPECFRCRACNLPISDYEFSTSGNYPYHKSCYKESYHPKCDVCKHFIPTNPAGLIEYRAHPFWIQKYCPTHEHDGTTRCCSCERMESQEAGYIALKDGRKLCLECLDSAIMDTNECQPLHADIQRFYESLNMKLDQQIPLLLVERQALNEAREGEKNGHYHMPETRGLCLSEELSTFSRRPRLGTTMDMRAQPYRPTTRCDVTAILILYGLPRLLTGSILAHEMMHAWLRLKGYRTLSQDVEEGICQVLSHMWLESELSSASGSNFVSASSSSASHTSRKGKRPQFERKLGEFFKHQIESDISPVYGGGFRAGQKAVSKYGLQRTLHHIRMTGTFPY

SEQ ID NO: 49 - protein, 462 aa, Vitis vinifera
MGWLNKIFKGSSHKISEGNYHGRYQGDTVQNEPSCSGDVWAETENEDIDRAIALSLSEEEQKGKKVIDNEFQLEEDEQLARAIQESLNIESPPQHGNGNGNGNIYQPIPFPYSTGFRICAGCNTEIGHGRFLSCMGAVWHPECFRCHGCGYPISDYEYSMNGNYPYHKSCYKEHYHPKCDVCKHFIPTNPAGLIEYRAHPFWVQKYCPSHEHDRTPRCCSCERMEPRDTRYVALNDGRKLCLECLDSAIMDTNECQPLYLDIQEFYEGLNMKVQQQVPLLLVERQALNEAMEGEKSGHHHMPETRGLCLSEEQTVSTILRRPKIGTGNRVMNMITEPCKLTRRCDVTAVLILYGLPRLLTGSILAHEMMHAWLRLNGYRTLAQDVEEGICQVLAYMWLDAELTSGSGRSQCERKLGQFFKHQIESDTSLVYGAGFRAGHQAVLKYGLPATLKHIHLTGNFPY

SEQ ID NO: 50 - protein, 482 aa, Vitis vinifera
MGWLNKIFKGSSHKISEGNYHGRYQGDTVQNEPSCSGDVWAETENEDIDRAIALSLSEEEQKGKKVIDELDNEFQLEEDEQLARAIQESLNIESPPQHGNGNGNGNIYQPIPFPYSTGFRICAGCNTEIGHGRFLSCMGAVWHPECFRCHGCGYPISDYEYSMNGNYPYHKSCYKEHYHPKCDVCKHFIPTNPAGLIEYRAHPFWVQKYCPSHEHDRTPRCCSCERMEPRDTRYVALNDGRKLCLECLDSAIMDTNECQPLYLDIQEFYEGLNMKVQQQVPLLLVERQALNEAMEGEKSGHHHMPETRGLCLSEEQTVSTILRRPKIGTGNRVMNMITEPCKLTRRCDVTAVLILYGLPRLLTGSILAHEMMHAWLRLNGYRTLAQDVEEGICQVLAYMWLDAELTSGSGSNVPSTSSASTSSKKGAGSQCERKLGQFFKHQIESDTSLVYGAGFRAGHQAVLKYGLPATLKHIHLTGNFPY

SEQ ID NO: 51 - protein, 486 aa, Solanum lycopersicum
MGWLNKIFRGSSHKISEGQYDWRCEGHTEEDDPSTAEDSWSEIEEIDRAIAISLSEEEQKGKIVIDSESQLKEDEQLARALQESLNVESPPQHVSRNDHGGGNVYGNGNFYHPVPFPYSASFRVCAGCSTEIGHGRFLSCMGAVWHPECFRCHACNQPISDYEFSMSGNYPYHKTCYKEHYHPKCDVCKHFIPTNAAGLIEYRAHPFWSQKYCPFHEHDGTPRCCSCERMEPRDTRYIALDDGRKLCLECLDSAIMDTSQCQPLYYDIQEFYEGLNMKVEQKVPLLLVERQALNEAMDGERHGYHHMPETRGLCLSEEQTISTIQRRPRIGAGNRVMDMRTEPYKLTRRCEVTAILILYGLPRLLTGSILAHEMMHAWLRLRGYRTLSQDVEEGICQVLAHMWLETQIASISSSNGGASTSSGMSSSKQGIRSPFERKLGDFFKHQIESDTSPIYGNGFRAGNQAVLKYGLERTLDHIRMTGTFPY

SEQ ID NO: 52 - protein, 878 aa, Oryza sativa
MGDRPDMGAGVALRFSHNDWTLEEDSKALHFLQPDLVLFTGDYGNENVQLVKSISDLQLPKAAILGNHDCWHTYQFSEKKVDRVQLQLESLGEQHVGYKCLDFPTIKLSVVGGRPFSCGGNRIFRPKLLSKWYGVNDMAESAKRIYDAATNAPKEHAVILLAHNGPTGLGSRMEDICGRDWVAGGGDHGDPDLEQAISDLQRETGVSIPLVVFGHMHKSLAYGRGLRKMIAFGANRTIYLNGAVVPRVNHAQSSRQPAISTSEKTGLEGLTGLMVPTSRAFTIVDLFEGAVEKISEVWVTVGDARTELEQELVLYKQPHKSVPSNIAIWSTMGWLTKFFRGSTHKISEGQYHSKPAEETIWNGPSNSAVVTMVYPLESTFGQLDLLLLATDLRQLVIDDVDCCKLRQQAQPVLHLMYSQLQLLQTSHAHQHGDVPSEFDNEDIARAISLSLLEEEQRKAKAIEKDMHLEEDEQLARAIQESLNVESPPRARENGNANGGNMYQPLPFMFSSGFRTCAGCHSEIGHGRFLSCMGAVWHPECFRCHACNQPIYDYEFSMSGNHPYHKTCYKERFHPKCDVCKQFIPTNMNGLIEYRAHPFWLQKYCPSHEVDGTPRCCSCERMEPRESRYVLLDDGRKLCLECLDSAVMDTSECQPLYLEIQEFYEGLNMKVEQQVPLLLVERQALNEAMEGEKTGHHHLPETRGLCLSEEQTVSTILRRPRMAGNKVMEMITEPYRLTRRCEVTAILILYGLPRLLTGSILAHEMMHAWLRLKGYRTLSPDVEEGICQVLAHMWIESEIIAGSGSNGASTSSSSSASTSSKKGGRSQFERKLGDFFKHQIESDTSMAYGDGFRAGNRAVLQYGLKRTLEHIRLTGTFPF

SEQ ID NO: 53 - protein, 486 aa, Oryza sativa
MGWLTKFFRGSTHKISEGQYHSKPAEETIWNGPSNSAVVTDVPSEFDNEDIARAISLSLLEEEQRKAKAIEKDMHLEEDEQLARAIQESLNVESPPRARENGNANGGNMYQPLPFMFSSGFRTCAGCHSEIGHGRFLSCMGAVWHPECFRCHACNQPIYDYEFSMSGNHPYHKTCYKERFHPKCDVCKQFIPTNMNGLIEYRAHPFWLQKYCPSHEVDGTPRCCSCERMEPRESRYVLLDDGRKLCLECLDSAVMDTSECQPLYLEIQEFYEGLNMKVEQQVPLLLVERQALNEAMEGEKTGHHHLPETRGLCLSEEQTVSTILRRPRMAGNKVMEMITEPYRLTRRCEVTAILILYGLPRLLTGSILAHEMMHAWLRLKGYRTLSPDVEEGICQVLAHMWIESEIIAGSGSNGASTSSSSSASTSSKKGGRSQFERKLGDFFKHQIESDTSMAYGDGFRAGNRAVLQYGLKRTLEHIRLTGTFPF

SEQ ID NO: 54 - protein, 512 aa, Brachypodium distachyon
MGWLTKIFRGSTYKISEGQRQSRPAEEAVWNEPSSSTVVTDVLSEFDNEDIDRAIALSLSEEQRKSKGTGKDLHLDEDEQLARAIHESLNVESPPCARDNGSPPHARDNSSPPHARENSSHPRARENGIANGGNSIQHSPFMFSSGFRTCAGCHSEIGHGRFLSCMGAVWHPECFCCHACSQPIYDYEFSMSGNHPYHKTCYKERFHPKCDVCKQFIPTNMNGLIEYRAHPFWLQKYCPSHEVDGTPRCCSCERMEPRESRYVLLDDGRKLCLECLDSAVMDTTECQPLYLEIQEFYEGLNMKVEQQVPLLLVERQALNEAMEGEKTGHHHLPETRGLCLSEEQTVSTILRRPRMTGNKIMEMITEPYRLTRRCEVTAILILYGLPRLLTGSILAHEMMHAWLRLKGYRTLSPEIEEGICQVLAHMWIESEIMAGSSSNAASTSSSSSSSISSKKGGRSQFERKLGDFFKHQIESDTSVAYGNGFRSGNQAVLQYGLKRTLEHIWLTGTWPF

SEQ ID NO: 55 - protein, 491 aa, Brachypodium distachyon
MGWLTKFFRGSTHNISEGQDQSKPAEETVWNEPSSSTAVNYALSEFDNEDIDRAIALSLSEEEQRKSKGTGKDQHLDEDEQLARAIQESLNVESPPRAREKSSHPRARENGSANGGNSYQLPLMFSSGFRTCAGCHSEIGHGRFLSCMGAVWHPECFCCHGCSQPIYDYEFSMSGNHPYHKTCYKERFHPKCDVCQQFIPTNTNGLIEYRAHPFWLQKYCPSHEVDGTPRCCSCERMEPRESRYVLLDDGRKLCLECLDSAVMDTTECQPLYLEIQEFYEGLNMKVEQQVPLLLVERQALNEAMEGEKTGHHHLPETRGLCLSEEQTVSTILRRPRMAGNKIMEMRTEPYRLTRRCEVTAILILYGLPRLLTGSILAHEMMHAWLRLKGYRTLSPDIEEGICQVLAHMWIESEITAGSGSNAASTSSSSTSSKKGGRSQFERKLGDFFKHQIESDTSVAYGDGFRAGNQAVLQYGLKRTLEHIRLTGTLPF

SEQ ID NO: 56 - protein, 486 aa, Sorghum bicolor
MGWLTKFFRGSTHNISEGQYHSRPAEDTAWNEPSSSPVVTDIFSEFNNEDIDRAIALSLSEEEQRKAKTIDKDMHLEEDEQLARAIQESLNVESPPPSRENGSANGGNAYHPLPFMFSSGFRACAGCHREIGHGRFLSCMGAVWHPECFRCHACSQPIYDYEFSMSGNHPYHKTCYKEQFHPKCDVCKQFIPTNMNGLIEYRAHPFWLQKYCPSHEVDGTPRCCSCERMEPRESRYVLLDDGRKLCLECLDSAVMDTNECQPLYLEIQEFYEGLNMKVEQQVPLLLVERQALNEAMEGEKAGHHHLPETRGLCLSEEQTVSTILRRPRMAGNKIMGMITEPYRLTRRCEVTAILILYGLPRLLTGSILAHEMMHAWLRLKGYRTLSPDVEEGICQVLAHLWIESEIMAGSGSGAASSSSGSSSSMSSKKAGRSQFEHKLGDFFKHQIETDTSMAYGEGFRAGNRAVLQYGLKRTLEHIRLTGTFPF

SEQ ID NO: 57 - protein, 508 aa, Zea mays
MGWLTKFFRGSTHNISEEQYHSRPAEDTAWNEPSSSPVVTDILSEFNNEDIDRAIALSLSEEEQRKEKAIDKDMHLEEDEQLARAIQESLNVESPPRRNGSANGGTMYHPPRETGNAYQPPRENGSANGGNAYHPLPFMFSSGFRACAGCHREIGHGRFLSCMGAVWHPECFRCHACSQPIYDYEFSMSGNHPYHKTCYKEQFHPKCDVCKQFIPTNMNGLIEYRAHPFWVQKYCPSHEMDGTPRCCSCERMEPRESKYVLLDDGRKLCLECLDSAVMDTNDCQPLYLEIQEFYEGLNMKVEQQVPLLLVERQALNEAMEGEKAGHHHLPETRGLCLSEEQTVSTILRPRMAGNKIMGMITEPYRLTRRCEVTAILILYGLPRLLTGSILAHEMMHAWLRLKGYRTLSPDVEEGICQVLAHMWIESEIMAGSGSSAASSSSGSSSSTSSKKGGRSQFEHRLGDFFKHQIETDTSMAYGDGFRTGNRAVLHYGLKRTLEHIRLTGTFPF

SEQ ID NO: 58 - protein, 553 aa, Arabidopsis thaliana
MGWLTKILKGSSHKFSDGQCNGRYREDRNLEGPRYSAEGSDFDKEEIECAIALSLSEQEHVIPQDDKGKKIIEYKSETEEDDDDDEDEDEEYMRAQLEAAEEEERRVAQAQIEEEEKRRAEAQLEETEKLLAKARLEEEEMRRSKAQLEEDELLAKALQESMNVGSPPRYDPGNILQPYPFLIPSSHRICVGCQAEIGHGRFLSCMGGVWHPECFCCNACDKPIIDYEFSMSGNRPYHKLCYKEQHHPKCDVCHNFIPTNPAGLIEYRAHPFWMQKYCPSHERDGTPRCCSCERMEPKDTKYLILDDGRKLCLECLDSAIMDTHECQPLYLEIREFYEGLHMKVEQQIPMLLVERSALNEAMEGEKHGHHHLPETRGLCLSEEQTVTTVLRRPRIGAGYKLIDMITEPCRLIRRCEVTAILILYGLPRLLTGSILAHEMMHAWLRLNGYPNLRPEVEEGICQVLAHMWLESETYAGSTLVDIASSSSSAVVSASSKKGERSDFEKKLGEFFKHQIESDSSSAYGDGFRQGNQAVLKHGLRRTLDHIRLTGTFP

SEQ ID NO: 59 - protein, 528 aa, Arabidopsis thaliana
MDSSSSSSSSSPSSSYGVARVSHISNPCIFGEVGSSSSSTYRDKKWKLMKWVSKLFKSGSNGGGSGAHTNHHPPQFQEDENMVFPLPPSSLDDRSRGARDKEELDRSISLSLADNTKRPHGYGWSMDNNRDFPRPFHGGLNPSSFIPPYEPSYQYRRRQRICGGCNSDIGSGNYLGCMGTFFHPECFRCHSCGYAITEHEFSLSGTKPYHKLCFKELTHPKCEVCHHFIPTNDAGLIEYRCHPFWNQKYCPSHEYDKTARCCSCERLESWDVRYYTLEDGRSLCLECMETAITDTGECQPLYHAIRDYYEGMYMKLDQQIPMLLVQREALNDAIVGEKNGYHHMPETRGLCLSEEQTVTSVLRRPRLGAHRLVGMRTQPQRLTRKCEVTAILVLYGLPRLLTGAILAHELMHGWLRLNGFRNLNPEVEEGICQVLSYMWLESEVLSDPSTRNLPSTSSVATSSSSSFSNKKGGKSNVEKKLGEFFKHQIAHDASPAYGGGFRAANAAACKYGLRRTLDHIRLTGTFPL

SEQ ID NO: 60 - protein, 1613 aa, Arabidopsis thaliana
MEPPAARVTPSIKADCSHSVNIICEETVLHSLVSHLSAALRREGISVFVDACGLQETKFFSIKQNQPLTDGARVLVVVISDEVEFYDPWFPKFLKVIQGWQNNGHVVVPVFYGVDSLTRVYGWANSWLEAEKLTSHQSKILSNNVLTDSELVEEIVRDVYGKLYPAERVGIYARLLEIEKLLYKQHRDIRSIGIWGMPGIGKTTLAKAVFNHMSTDYDASCFIENFDEAFHKEGLHRLLKERIGKILKDEFDIESSYIMRPTLHRDKLYDKRILVVLDDVRDSLAAESFLKRLDWFGSGSLIIITSVDKQVFAFCQINQIYTVQGLNVHEALQLFSQSVFGINEPEQNDRKLSMKVIDYVNGNPLALSIYGRELMGKKSEMETAFFELKHCPPLKIQDVLKNAYSALSDNEKNIVLDIAFFFKGETVNYVMQLLEESHYFPRLAIDVLVDKCVLTISENTVQMNNLIQDTCQEIFNGEIETCTRMWEPSRIRYLLEYDELEGSGETKAMPKSGLVAEHIESIFLDTSNVKFDVKHDAFKNMFNLKFLKIYNSCSKYISGLNFPKGLDSLPYELRLLHWENYPLQSLPQDFDFGHLVKLSMPYSQLHKLGTRVKDLVMLKRLILSHSLQLVECDILIYAQNIELIDLQGCTGLQRFPDTSQLQNLRVVNLSGCTEIKCFSGVPPNIEELHLQGTRIREIPIFNATHPPKVKLDRKKLWNLLENFSDVEHIDLECVTNLATVTSNNHVMGKLVCLNMKYCSNLRGLPDMVSLESLKVLYLSGCSELEKIMGFPRNLKKLYVGGTAIRELPQLPNSLEFLNAHGCKHLKSINLDFEQLPRHFIFSNCYRFSSQVIAEFVEKGLVASLARAKQEELIKAPEVIICIPMDTRQRSSFRLQAGRNAMTDLVPWMQKPISGFSMSVVVSFQDDYHNDVGLRIRCVGTWKTWNNQPDRIVERFFQCWAPTEAPKVVADHIFVLYDTKMHPSDSEENHISMWAHEVKFEFHTVSGENNPLGASCKVTECGVEVITAATGDTSVSGIIRESETITIIEKEDTIIDEEDTPLLSRKPEETNRSRSSSELQKLSSTSSKVRSKGNVFWKWLGCFPLQPKNLRSRSRRTTALEEALEEALKEREKLEDTRELQIALIESKKIKKIKQADERDQIKHADEREQRKHSKDHEEEEIESNEKEERRHSKDYVIEELVLKGKGKRKQLDDDKADEKEQIKHSKDHVEEEVNPPLSKCKDCKSAIEDGISINAYGSVWHPQCFCCLRCREPIAMNEISDLRGMYHKPCYKELRHPNCYVCEKKIPRTAEGLKYHEHPFWMETYCPSHDGDGTPKCCSCERLEHCGTQYVMLADFRWLCRECMDSAIMDSDECQPLHFEIREFFEGLHMKIEEEFPVYLVEKNALNKAEKEEKIDKQGDQCLMVVRGICLSEEQIVTSVSQGVRRMLNKQILDTVTESQRVVRKCEVTAILILYGLPRLLTGYILAHEMMHAYLRLNGYRNLNMVLEEGLCQVLGYMWLECQTYVFDTATIASSSSSSRTPLSTTTSKKVDPSDFEKRLVNFCKHQIETDESPFFGDGFRKVNKMMASNNHSLKDTLKEIISISKTPQYSKL

SEQ ID NO: 61 - protein, 450 aa, Arabidopsis thaliana
MVRRKRQEEDEKIEIERVKEESLKLAKQAEEKRRLEESKEQGKRIQVDDDQLAKTTSKDKGQINHSKDVVEEDVNPPPSIDGKSEIGDGTSVNPRCLCCFHCHRPFVMHEILKKGKFHIDCYKEYYRNRNCYVCQQKIPVNAEGIRKFSEHPFWKEKYCPIHDEDGTAKCCSCERLEPRGTNYVMLGDFRWLCIECMGSAVMDTNEVQPLHFEIREFFEGLFLKVDKEFALLLVEKQALNKAEEEEKIDYHRAAVTRGLCMSEEQIVPSIIKGPRMGPDNQLITDIVTESQRVSGFEVTGILIIYGLPRLLTGYILAHEMMHAWLRLNGYKNLKLELEEGLCQALGLRWLESQTFASTDAAAAAAVASSSSFSSSTAPPAAITSKKSDDWSIFEKKLVEFCMNQIKEDDSPVYGLGFKQVYEMMVSNNYNIKDTLKDIVSASNATPDSTV

SEQ ID NO: 62 - protein, 702 aa, Arabidopsis thaliana
MPISDVASLVGGAALGAPLSEIFKLVIEEAKKVKDFKPLSQDLASTMERLVPIFNEIDMMQQGSNRGTSELKVLTETMERAGEMVHKCSRIQWYSIAKKALYTREIKAINQDFLKFCQIELQLIQHRNQLQYMRSMGMASVSTKADLLSDIGNEFSKLCLVAQPEVVTKFWLKRPLMELKKMLFEDGVVTVVVSAPYALGKTTLVTKLCHDADVKEKFKQIFFISVSKFPNVRLIGHKLLEHIGCKANEYENDLDAMLYIQQLLKQLGRNGSILLVLDDVWAEEESLLQKFLIQLPDYKILVTSRFEFTSFGPTFHLKPLIDDEVECRDEIEENEKLPEVNPPLSMCGGCNSAVKHEESVNILGVLWHPGCFCCRSCDKPIAIHELENHVSNSRGKFHKSCYERYCYVCKEKKMKTYNIHPFWEERYCPVHEADGTPKCCSCERLEPRGTKYGKLSDGRWLCLECGKSAMDSDECQPLYFDMRDFFESLNMKIEKEFPLILVRKELLNKKEEKIDNHYEVLIRAYCMSEQKIMTYVSEEPRTGQNKQLIDMDTEPQGVVHECKVTAILILYGLPRLLTGYILAHEMMHAWLRLNGHMNLNNILEEGICQVLGHLWLESQTYATADTTADAASASSSSSRTPPAASASKKGEWSDFDKKLVEFCKNQIETDESPVYGLGFRTVNEMVTNSSLQETLKEILRRR

SEQ ID NO: 63 - protein, 644 aa, Arabidopsis thaliana
MASDYYSSDDEGFGEKVGLIGEKDRFEAETIHVIEVSQHEADIQKAKQRSLATHEAEKLDLATHEAEQLDLAIQEFSRQEEEEERRRTRELENDAQIANVLQHEERERLINKKTALEDEEDELLARTLEESLKENNRRKMFEEQVNKDEQLALIVQESLNMEEYPIRLEEYKSISRRAPLDVDEQFAKAVKESLKNKGKGKQFEDEQVKKDEQLALIVQESLNMVESPPRLEENNNISTRAPVDEDEQLAKAVEESLKGKGQIKQSKDEVEGDGMLLELNPPPSLCGGCNFAVEHGGSVNILGVLWHPGCFCCRACHKPIAIHDIENHVSNSRGKFHKSCYERYCYVCKEKKMKTYNNHPFWEERYCPVHEADGTPKCCSCERLEPRESNYVMLADGRWLCLECMNSAVMDSDECQPLHFDMRDFFEGLNMKIEKEFPFLLVEKQALNKAEKEEKIDYQYEVVTRGICLSEEQIVDSVSQRPVRGPNNKLVGMATESQKVTRECEVTAILILYGLPRLLTGYILAHEMMHAYLRLNGHRNLNNILEEGICQVLGHLWLDSQTYATADATADASSSASSSSRTPPAASASKKGEWSDFDKKLVEFCKNQIETDDSPVYGLGFRTVNEMVTNSSLQETLKEILRQR

SEQ ID NO: 64 - protein, 587 aa, Arabidopsis thaliana
MWCLSCFKPSTKHDPSEDRFEEETNIVTGISLYEDVILRQRRSEADQIEWAIQDSFNPQETSRCRQREEDDQIARGLQYVEETELDKSVVDEEDQQLSKIVEESLKEKGKSKQFEDDQVENDEQQALMVQESLYMVELSAQLEEDKNISTIPPLNEDAQLQKVIWESAKGKGQIEHFKDPVEEDGNLPRVDLNVNHPHSICDGCKSAIEYGRSVHALGVNWHPECFCCRYCDKPIAMHEFSNTKGRCHITCYERSHPNCHVCKKKFPGRKYKEHPFWKEKYCPFHEVDGTPKCCSCERLEPWGTKYVMLADNRWLCVKCMECAVMDTYECQPLHFEIREFFGSLNMKVEKEFPLLLVEKEALKKAEAQEKIDNQHGVVTRGICLSEGQIVNSVFKKPTMGPNGELVSLGTEPQKVVGGCEVTAILILYGLPRLLTGYILAHEMMHAWLRLNGTTSTQFVFANQYGESSQLKVLFGLITGYRNLKLELEEGICQVLGHMWLESQTYSSSAAASSASSSSRTPAANASKKGAQSDYEKKLVEFCKDQIETDDSPVYGVGFRKVNQMVSDSSLHKILKSIQHWTKPDSNL

SEQ ID NO: 65 - protein, 5 aa, Artificial sequence
  Synthetic sequence: Metallopetidase motif
HEMMH

SEQ ID NO: 66 - protein, 19 aa, Artificial sequence
  Synthetic sequence: Carboxyl terminal region motif
  VARIANT (3)..(10): Xaa is any amino acid
  VARIANT (12)..(15): Xaa is any amino acid
EKXXXXXXXXRXXXXSEEQ

SEQ ID NO: 67 - protein, 18 aa, Artificial sequence
  Synthetic sequence: Carboxyl terminal region motif
  VARIANT (3)..(10): Xaa is any amino acid
  VARIANT (12)..(15): Xaa is any amino acid
EKXXXXXXXXRXXXXSEQ

SEQ ID NO: 68 - protein, 21 aa, Artificial sequence
  Synthetic sequence: UIM1 domain
  VARIANT (1)..(1): Xaa is a polar amino acid residue, for example Cys, Asp, Glu, His, Lys, Asn, Gln, Arg, Ser or Thr
  VARIANT (2)..(4): Xaa is any amino acid
  VARIANT (5)..(5): Xaa is a polar amino acid residue, for example Cys, Asp, Glu, His, Lys, Asn, Gln, Arg, Ser or Thr
  VARIANT (7)..(7): Xaa is a polar amino acid residue, for example Cys, Asp, Glu, His, Lys, Asn, Gln, Arg, Ser or Thr
  VARIANT (8)..(8): Xaa is a big amino acid residue, for example Glu, Phe, His, Ile, Lys, Met, Gln, Arg, Trp or Tyr
  VARIANT (10)..(10): Xaa is an aliphatic amino acid residue, for example Ile, Leu or Val
  VARIANT (11)..(11): Xaa is a polar amino acid residue, for example Cys, Asp, Glu, His, Lys, Asn, Gln, Arg, Ser or Thr
  VARIANT (12)..(12): Xaa is a big amino acid residue, for example Glu, Phe, His, Ile, Lys, Met, Gln, Arg, Trp or Tyr
  VARIANT (13)..(13): May be present or absent. If present, Xaa is any amino acid.
  VARIANT (15)..(15): Xaa is a big amino acid residue, for example Glu, Phe, His, Ile, Lys, Met, Gln, Arg, Trp or Tyr
  VARIANT (16)..(16): Xaa is a polar amino acid residue, for example Cys, Asp, Glu, His, Lys, Asn, Gln, Arg, Ser or Thr
  VARIANT (17)..(17): Xaa is any amino acid
  VARIANT (18)..(18): May be present or absent. If present, Xaa is any amino acid.
  VARIANT (19)..(21): Xaa is a polar amino acid residue, for example Cys, Asp, Glu, His, Lys, Asn, Gln, Arg, Ser or Thr
XXXXXLXXAXXXXSXXXXXXX

SEQ ID NO: 69 - protein, 21 aa, Artificial sequence
  Synthetic sequence: UIM2 domain
  VARIANT (1)..(1): Xaa is a polar amino acid residue, for example Cys, Asp, Glu, His, Lys, Asn, Gln, Arg, Ser or Thr
  VARIANT (2)..(4): Xaa is any amino acid
  VARIANT (5)..(5): Xaa is a polar amino acid residue, for example Cys, Asp, Glu, His, Lys, Asn, Gln, Arg, Ser or Thr
  VARIANT (7)..(7): Xaa is a polar amino acid residue, for example Cys, Asp, Glu, His, Lys, Asn, Gln, Arg, Ser or Thr
  VARIANT (8)..(8): Xaa is a big amino acid residue, for example Glu, Phe, His, Ile, Lys, Met, Gln, Arg, Trp or Tyr
  VARIANT (10)..(10): Xaa is an aliphatic amino acid residue, for example Ile, Leu or Val
  VARIANT (11)..(11): Xaa is a polar amino acid residue, for example Cys, Asp, Glu, His, Lys, Asn, Gln, Arg, Ser or Thr
  VARIANT (12)..(12): Xaa is a big amino acid residue, for example Glu, Phe, His, Ile, Lys, Met, Gln, Arg, Trp or Tyr
  VARIANT (13)..(13): May be present or absent. If present, Xaa is any amino acid.
  VARIANT (15)..(15): Xaa is a big amino acid residue, for example Glu, Phe, His, Ile, Lys, Met, Gln, Arg, Trp or Tyr
  VARIANT (16)..(16): Xaa is a polar amino acid residue, for example Cys, Asp, Glu, His, Lys, Asn, Gln, Arg, Ser or Thr
  VARIANT (17)..(17): Xaa is any amino acid
  VARIANT (18)..(18): Xaa is a small amino acid residue, for example Ala, Cys, Asp, Gly, Asn, Pro, Ser, Thr or Val
  VARIANT (19)..(21): Xaa is a polar amino acid residue, for example Cys, Asp, Glu, His, Lys, Asn, Gln, Arg, Ser or Thr
XXXXXLXXAXXXXSXXXXXXX

SEQ ID NO: 70 - protein, 20 aa, Artificial sequence
  Synthetic sequence: UIM1 domain
QENEDIDRAIALSLLEENQE

SEQ ID NO: 71 - protein, 20 aa, Artificial sequence
  Synthetic sequence: UIM2 domain
DEDEQIARALQESMVVGNSP

SEQ ID NO: 72 - protein, 53 aa, Artificial sequence
  Synthetic sequence: LIM domain
ICAGCNMEIGHGRFLNCLNSLWHPECFRCYGCSQPISEYEFSTSGNYPFHKAC

SEQ ID NO: 73 - protein, 43 aa, Artificial sequence
  Synthetic sequence: EOD domain
  VARIANT (1)..(1): Xaa is Glu or Lys
  VARIANT (8)..(8): Xaa is Leu or Met
  VARIANT (9)..(9): Xaa is Lys, Arg, Gly, Thr or Glu
  VARIANT (11)..(11): Xaa is Lys or Arg
  VARIANT (12)..(12): Xaa is Arg or Ile
  VARIANT (13)..(13): Xaa is Gly or Lys
  VARIANT (14)..(14): Xaa is Asp, Asn or Glu
  VARIANT (15)..(15): Xaa is Arg, Gln, Lys or Leu
  VARIANT (17)..(17): Xaa is Ile, Met or Val
  VARIANT (18)..(18): Xaa is Lys, Asn, Thr or Ala
  VARIANT (20)..(20): Xaa is Leu or Pro
  VARIANT (22)..(22): Xaa is Lys or Ser
  VARIANT (24)..(24): Xaa is Val or Ala
  VARIANT (27)..(27): Xaa is Ser, Thr, Gly or Ala
  VARIANT (28)..(28): Xaa is Glu, Gln, Asp, Ser or Gly
  VARIANT (30)..(30): Xaa is Ile, Gly, Thr or Val
  VARIANT (31)..(31): Xaa is Ser or Thr
  VARIANT (32)..(32): Xaa is Lys or Arg
  VARIANT (35)..(35): Xaa is Gly, Thr or Ser
  VARIANT (39)..(39): Xaa is Val, Ile, Ala or Lys
  VARIANT (42)..(42): Xaa is Val or Ile
XRCVICQXXYXXXXXQXXLXCXHXYHXXCXXXWLXINKXCPXC

SEQ ID NO: 74 - protein, 253 aa, Zea mays
MNSSRQMELHYINTGFPYTITESFMDFFEGLTYAHADFALTDGFQDQGNPYWAMMHTNSYKYGYSGPGNYYSYAHVYDIDDYMRRADGGRRIWDNTTPVNNVDSANVVLQGGEAPHTTTNTINKECIQQVHQSPGSPQVVWQDNIEPDNMTYEELLDLGEAVGTQSRGLSQERISSLPVTKYKCGFFSRKKTRRERCVICQMEYRRGNLQMTLPCKHVYHASCVTRWLGINKVCPVCFAEVPGEDPEAMSQQL

SEQ ID NO: 75 - protein, 249 aa, Sorghum bicolor
MNSCRQMELHYINTGFPYTITESFMDFFEGLTYAHADFALMDGFQDQGNPYWAMMHTNSYKYGYSGPGNYYTYAHVYDIDDYMHRADGGRRVWDNTTPANNVDSANVVLQGSEAPRTTANTTTEECIQQVHQSPGSPHVVWQDNIDPDNMTYEELLDLGEVVGTQSRGLSQERISSLPVTKYKCGFFSRKKTRRERCVICQMEYRRGNLQMTLPCKHVYHASCVTRWLSINKVCPVCFAEVPGDEPKRQ

SEQ ID NO: 76 - protein, 249 aa, Zea mays
MTSSRQMELHYINTGFPYTITESFMDFFEGLTYAHADFALMDGFQDQGNPYWTMMHTNSYKYGYSGSGNYYSYAHAYDIDDYMHRTDGGRRTWDNTTPVNNVDSANVVLQGGEAPRTTANTTSEDCIQQVHQSPGSPQVVWQDNIDPDNMTYEELLDLGEAVGTQSRGLSQECISLLPITKYKCGFFSRKKTRRERCVICQMEYRRGNLQITLPCKHVYHASCVTRWLSINKVCPVCFAEVPGEDSLRQ

SEQ ID NO: 77 - protein, 272 aa, Oryza sativa
MTESHERDTEVTRWQVHDPSEGMNGSRQMELHYINTGFPYTITESFMDFFEGLTYAHADFAIADAFHDQANPYWAMMHTNSYKYGYSGAGNYYSYGHVYDMNDYMHRADGGRRIWDNATPVNNTESPNVVLQGGETPHANTSSTTEECIQQQVHQNSSSPQVIWQDNIDPDNMTYEELLDLGEAVGTQSRGLSQERISLLPVTKYKCGFFSRKKTRRERCVICQMEYRRGNLQMTLPCKHVYHASCVTRWLSINKVCPVCFAEVPGDEPKRQ

SEQ ID NO: 78 - protein, 250 aa, Oryza sativa
MNGSRQMELHYINTGFPYTITESFMDFFEGLTYAHADFAIADAFHDQANPYWAMMHTNSYKYGYSGAGNYYSYGHVYDMNDYMHRADGGRRIWDNATPVNNTESPNVVLQGGETPHANTSSTTEECIQQQVHQNSSSPQVIWQDNIDPDNMTYEELLDLGEAVGTQSRGLSQERISLLPVTKYKCGFFSRKKTRRERCVICQMEYRRGNLQMTLPCKHVYHASCVTRWLSINKVCPVCFAEVPGDEPKRQ

SEQ ID NO: 79 - protein, 251 aa, Brachypodium distachyon
MNGSRQMELHYINTGFPYTITESFMDFFEGLTYAHADFALADAFQDQANPYWTMMQTNSYKYGYSGASNYYSYGHVYDMNDYMHRADGGRRIWDNPTPASNTDSPNVVLQGAAEAPHPRASSTTEECIQQPVHQNSSSPQVVWQDNVDPDNMTYEELLDLGEAVGTQSRGLSQERISSLPVTKYKCGFFSRKKTRRERCVICQMEYRRGDLQMALPCKHVYHASCVTRWLSINKVCPVCFAEVPSEEPSRQ

SEQ ID NO: 80 - protein, 246 aa, Solanum lycopersicum
MNWNQQTEIYYTNGAMPYNSIGSFMDFFGGVTYDHVNYIFADPPYAQESLYPSISTNPYKFGYSEAGSFSYYDYDREYVVNDHVSGIEEHDRHLENPSTTTVNVAANVHREEISGSNSLTNSVECPRGQINTRDSEVVWQDNIDPDNMTYEELLELGEAVGTQSRGLSQNQISLLPVTKFKCGFFSRKKSRKERCVICQMEYKRKDQQVTLPCKHVYHAGCGSRWLSINKACPICYTEVVINTSKR

SEQ ID NO: 81 - protein, 240 aa, Ricinus communis
MEVHYINTGFPYTVTESFLDFFEGLSHVPVHYAHTGQVLDQVQENAYWSMNMNAYKYGFSGPGSTYYDPYEVNDNLPRMDVSRSTWEYPSVVNMEEATTTDTQSEGDAVVGVHASPEECIPNHTSGDSPQGVWQDDVDPDNMTYEELLDLGETVGTQSRGLSQELISLLPTSKCKFRSFFLRKKAGERCVICQMRYKRGDKQMKLPCKHVYHSECISKWLGINKVCPVCNNEVFGEDSRH

SEQ ID NO: 82 - protein, 203 aa, Populus trichocarpa
MEVHYMNTDFPYTTTESFMDFFEGLTHAPVNYAHNGPMHDQDNAYWSMNMNAYKFGFSGLGSTSYYSPYEVNDNLPRMDVSRMAWEYPSVVIKALWQDDVDPDTMTYEELVDLGETVGTQSKGLSPELISLLPTSKCKFGSFFSRKRSGERCVICQMKYKRGDKQIKLLCKHAYHSECITKWLGINKVCPVCNDEVFGEESRN

SEQ ID NO: 83 - protein, 247 aa, Glycine max
MNDGRQMGVHYVDAGFPYAVNDNFVDFFQGFTHVPVNYAFAGSIPDQESVYWSMNMNPYKFGLSGPGSTSYYSSYEVNGHLPRMEIDRAEWEYPSTITTVEEPATTDSPPRRDGVTSMQTIPEECSPNHHESNSSSQVIWQDNIYPDDMTYEELLDLGEAVGTQSRGLSQELIDMLPTSKYKFGSLFKRKNSGKRCVICQMTYRRGDQQMKLPCSHVYHGECITKWLSINKKCPVCNTEVFGEESTH

SEQ ID NO: 84 - protein, 247 aa, Glycine max
MNDGRQMGVNYVDAGFPYAVNENFVDFFQGFTPVPVNYAFAGSIPDQESVYWSMNMNPYKFGLSGPGSTSYYSSYEVNGHLPRMEIDRAEWEYPSTITTVEEPATTDSPPRRDGVTNMQTIPEECSPNHHESNSSSQVIWQDNIDPDNMTYEELLDLGEAVGTQSRGLSQELIDMLPTSKYKFGNLFKRKNSGKRCVICQMTYRRGDQQMKLPCSHVYHGECITKWLSINKKCPVCNTEVFGEESTH

SEQ ID NO: 85 - protein, 247 aa, Vitis vinifera
MNGNRQMEVHYINTGFPYTITESFMDFFEGLGHVPVNYAQAEAMHNQSIQENFYWTMNMNSYKFGFSGPGSTYYGPYDVNEHVPGIEVSRRPWEYPSSMIVEEPTTIETQPTGNEVMNVHAIPEECSPNHYSATSSQAIWQDNVDPDNMTYEELLDLGEAVGTQSRGLSQEHINLLPTCRYKSGRLFSRKRSAERCVICQMGYKRGDRQIKLPCKHVYHTDCGTKWLTINKVCPVCNIEVFGEESRH

SEQ ID NO: 86 - protein, 242 aa, Theobroma cacao
MNGNRQMEVHYIDTGFPYTATESFMDFFEGLTHVPVNYTHTVPMQDQENIYWSMSMNAYKFGFSGPESTFYSPYEVSDHLPRMDVSRRTWDYPSTLNSEEPATIDMQPGGEAVVGIHAIPEECITNHQSNSNSQVVWQDNIDPDNMTYEELLDLGETIGSQSRGLSQELIDLLPTSKCKFGSFFSTKRERCVICQMRYKRGEQQMKLPCKHVYHSQCITKWLSINKICPVCNNEVFGEESRH

SEQ ID NO: 87 - protein, 245 aa, Prunus persica
MNGNGQMDVHYIDTDFPYTPTESFMDFFGGVTHVPMNYGHAMPMHDQETAYWSMNMHSYKFGPSGPGSNSYYGNYYEVNDHLPRMDVSRRTWEHPSVMNSEEPANIDSHPEEEDAVAEAAPEECIQNQQNTNTSQVVWQEDIDPDNMTYEELLDLGEAVGTQSRGLSDELISLLPTSKYKCGSFFSRKKSGERCVICQMRYKRGDRQINLPCKHVYHSECISKWLGINKVCPVCNLEVSGEESRH

SEQ ID NO: 88 - protein, 243 aa, Capsella rubella
MNGDRPVEDAHYTEAEFPYAASGSYIDFYGGAPQGPLNYAHAGTMDNLYWTMNTNAYKFGFSGSDNPSFYNSYDMTDHLSRMSIGRTNWEYHPMVNVDDPDITLARSVQIGDSDEHSEAEDCIANEHDPDSPQVSWQDDIDPDTMTYEELVELGEAVGTESRGLSQELIETLPTRKFKFGSIFSRKRAGERCVICQLKYKIGERQMNLPCKHVYHSECISKWLSINKVCPVCNTEVFGDPSIH

SEQ ID NO: 89 - protein, 248 aa, Arabidopsis thaliana
MNGDNRPVEDAHYTETGFPYAATGSYMDFYGGAAQGPLNYDHAATMHPQDNLYWTMNTNAYKFGFSGSDNASFYGSYDMNDHLSRMSIGRTNWDYHPMVNVADDPENTVARSVQIGDTDEHSEAEECIANEHDPDSPQVSWQDDIDPDTMTYEELVELGEAVGTESRGLSQELIETLPTKKYKFGSIFSRKRAGERCVICQLKYKIGERQMNLPCKHVYHSECISKWLSINKVCPVCNSEVFGEPSIH

SEQ ID NO: 90 - protein, 243 aa, Solanum lycopersicum
MSGDQHMEAMHYMNMGFPYNVPESFPGFLDGVSQAPIIQYHNNPVQIQDQENAYWSMNMSYYKYEHSNLESTSYHSYETGNNHVSRPDFSERPWEYAVPMNVHEGVSTDVIYEENTVPVEDVGTEECVLSNQDDSNHQDILEDEIDLDNMTYEELLDLGETVGTESRGLAEELINLLPTTKYKSNGIFSRKKSEERCVICQMRYKRGDRQINFPCKHIYHTECGSKWLSINKRCSLMNEVVQW

SEQ ID NO: 91 - protein, 10 aa, Artificial sequence
  Synthetic sequence: LIM domain
  VARIANT (2)..(3): Xaa is any amino acid
  VARIANT (5)..(6): Xaa is any amino acid
  VARIANT (8)..(9): Xaa is any amino acid
HXXCXXCXXC